European Patent Specification EP 3 469 362 B1, published December 4, 2024. Title: HUMAN LEUKOCYTE ANTIGEN RESTRICTED GAMMA DELTA T CELL RECEPTORS AND METHODS OF USE THEREOF. Applicant: UMC UTRECHT HOLDING B.V. The sequence listing filed with the application follows.

SEQUENCE LISTING (444 sequences)

SEQ ID NO: 1 - DNA, 3416 bp, Homo sapiens
gagaagccaatcagtgtcgtcgcggtcgctgttctaaagtccgcacgcacccaccgggactcagattctccccagacgccgaggatggccgtcatggcgccccgaaccctcctcctgctactctcgggggccctggccctgacccagacctgggcgggtgagtgcggggtcgggagggaaaccgcctctgcggggagaagcaaggggccctcctggcgggggcgcaggaccgggggagccgcgccgggaggagggtcgggcaggtctcagccactgctcgcccccaggctcccactccatgaggtatttcttcacatccgtgtcccggcccggccgcggggagccccgcttcatcgccgtgggctacgtggacgacacgcagttcgtgcggttcgacagcgacgccgcgagccagaagatggagccgcgggcgccgtggatagagcaggaggggccggagtattgggaccaggagacacggaatatgaaggcccactcacagactgaccgagcgaacctggggaccctgcgcggctactacaaccagagcgaggacggtgagtgaccccggcccggggcgcaggtcacgacccctcatcccccacggacgggccaggtcgcccacagtctccgggtccgagatccaccccgaagccgcgggactccgagacccttgtcccgggagaggcccaggcgcctttacccggtttcattttcagtttaggccaaaaatccccccgggttggtcggggcggggcggggctcgggggactgggctgaccgcggggtcggggccaggttctcacaccatccagataatgtatggctgcgacgtggggccggacgggcgcttcctccgcgggtaccggcaggacgcctacgacggcaaggattacatcgccctgaacgaggacctgcgctcttggaccgcggcggacatggcagctcagatcaccaagcgcaagtgggaggcggtccatgcggcggagcagcggagagtctacctggagggccggtgcgtggacgggctccgcagatacctggagaacgggaaggagacgctgcagcgcacgggtaccaggggccacggggcgcctccctgatcgcctatagatctcccgggctggcctcccacaaggaggggagacaattgggaccaacactagaatatcaccctccctctggtcctgagggagaggaatcctcctgggtttccagatcctgtaccagagagtgactctgaggttccgccctgctctctgacacaattaagggataaaatctctgaaggagtgacgggaagacgatccctcgaatactgatgagtggttccctttgacaccggcagcagccttgggcccgtgacttttcctctcaggccttgttctctgcttcacactcaatgtgtgtgggggtctgagtccagcacttctgagtctctcagcctccactcaggtcaggaccagaagtcgctgttcccttctcagggaatagaagattatcccaggtgcctgtgtccaggctggtgtctgggttctgtgctctcttccccatcccgggtgtcctgtccattctcaagatggccacatgcgtgctggtggagtgtcccatgacagatgcaaaatgcctgaattttctgactcttcccgtcagacccccccaagacacatatgacccaccaccccatctctgaccatgaggccaccctgaggtgctgggccctgggcttctaccctgcggagatcacactgacctggcagcgggatggggaggaccagacccaggacacggagctcgtggagaccaggcctgcaggggatggaaccttccagaagtgggcggctgtggtggtgccttctggagaggagcagagatacacctgccatgtgcagcatgagggtctgcccaagcccctcaccctgagatggggtaaggagggagatgggggtgtcatgtctcttagggaaagcaggagcctctctggagacctttagcagggtcagggcccctcaccttcccctcttttcccagagctgtcttcccagcccaccatccccatcgtgggcatcattgctggcctggttctccttggagctgtgatcactggagctgtggtcgctgccgtgatgtggaggaggaagagctcaggtggagaaggggtgaagggtggggtctgagatttcttgtctcactgagggttccaagccccagctagaaatgtgccctgtctcattactgggaagcaccttccacaatcatgggccgacccagcctgggccctgtgtgccagcacttactcttttgtaaagcacctgttaaaatgaaggacagatttatcaccttgattacggcggtgatgggacctgatcccagcagtcacaagtcacaggggaaggtccctgaggacagacctcaggagggctattggtccaggacccacacctgctttcttcatgtttcctgatcccgccctgggtctgcagtcacacatttctggaaacttctctggggtccaagactaggaggttcctctaggaccttaaggccctggctcctttctggtatctcacaggacattttcttcccacagatagaaaaggagggagttacactcaggctgcaagtaagtatgaaggaggctgatgcctgaggtccttgggatattgtgtttgggagcccatgggggagctcacccaccccacaattcctcctctagccacatcttctgtgggatctgaccaggttctgtttttgttctaccccaggcagtgacagtgcccagggctctgatgtgtctctcacagcttgtaaaggtgagagcttggagggcctgatgtgtgttgggtgttgggtggaacagtggacacagctgtgctatggggtttctttgcgttggatgtattgagcatgcgatgggctgtttaaggtgtgacccctcactgtgatggatatgaatttgttcatgaatatttttttctatagtgtgagacagctgccttgtgtgggactgagaggcaagagttgttcctgcccttccctttgtgacttgaagaaccctgactttgtttctgcaaaggcacctgcatgtgtctgtgttcgtgtaggcataatgtgaggaggtggggagagcaccccacccccatgtccaccatgaccctcttcccacgctgacctgtgctccctctccaatcatctttcctgttccagagaggtggggctgaggtgtctccatctctgtctcaacttcatggtgcactgagctgtaacttcttccttccctattaaaattagaacctgagtataaatttactttctcaaattcttgccatgagaggttgatgagttaattaaaggagaagattcctaaaatttgagagacaaaattaatggaacgcatgagaaccttccagagtcca

SEQ ID NO: 2 - protein, 15 aa, Artificial Sequence
  source: /note="Description of Artificial Sequence: Synthetic peptide"
CATWDRPEIYYKKLF

SEQ ID NO: 3 - protein, 19 aa, Artificial Sequence
  source: /note="Description of Artificial Sequence: Synthetic peptide"
CALGDSYGGGPLYTDKLIF

SEQ ID NO: 4 - protein, 309 aa, Artificial Sequence
  source: /note="Description of Artificial Sequence: Synthetic polypeptide"
MGWALLVLLAFLSPASQKSSNLEGGTKSVTRPTRSSAEITCDLTVINAFYIHWYLHQEGKAPQRLLYYDVSNSKDVLESGLSPGKYYTHTPRRWSWILILRNLIENDSGVYYCATWDRPEIYYKKLFGSGTTLVVTDKQLDADVSPKPTIFLPSIAETKLQKAGTYLCLLEKFFPDVIKIHWEEKKSNTILGSQEGNTMKTNDTYMKFSWLTVPEKSLDKEHRCIVRHENNKNGVDQEIIFPPIKTDVITMDPKDNCSKDANDTLLLQLTNTSAYYMYLLLLLKSVVYFAIITCCLLRRTAFCCNGEKS

SEQ ID NO: 5 - protein, 293 aa, Artificial Sequence
  source: /note="Description of Artificial Sequence: Synthetic polypeptide"
MVFSSLLCVFVAFSYSGSSVAQKVTQAQSSVSMPVRKAVTLNCLYETSWWSYYIFWYKQLPSKEMIFLIRQGSDEQNAKSGRYSVNFKKAAKSVALTISALQLEDSAKYFCALGDSYGGGPLYTDKLIFGKGTRVTVEPRSQPHTKPSVFVMKNGTNVACLVKEFYPKDIRINLVSSKKITEFDPAIVISPSGKYNAVKLGKYEDSNSVTCSVQHDNKTVHSTDFEVKTDSTDHVKPKETENTKQPSKSCHKPKAIVHTEKVNMMSLTVLGLRMLFAKTVAVNFLLTAKLFFL

SEQ ID NO: 6 - protein, 19 aa, Artificial Sequence
  source: /note="Description of Artificial Sequence: Synthetic peptide"
CALGDSYGGGPLYTDKLIF

SEQ ID NO: 7 - protein, 19 aa, Artificial Sequence
  source: /note="Description of Artificial Sequence: Synthetic peptide"
CALGESYGGGPLYTDKLIF

SEQ ID NO: 8 - protein, 19 aa, Artificial Sequence
  source: /note="Description of Artificial Sequence: Synthetic peptide"
CALGNSYGGGPLYTDKLIF

SEQ ID NO: 9 - protein, 19 aa, Artificial Sequence
  source: /note="Description of Artificial Sequence: Synthetic peptide"
CALGQSYGGGPLYTDKLIF

SEQ ID NO: 10 - protein, 19 aa, Artificial Sequence
  source: /note="Description of Artificial Sequence: Synthetic peptide"
CALGDTYGGGPLYTDKLIF

SEQ ID NO: 11 - protein, 19 aa, Artificial Sequence
  source: /note="Description of Artificial Sequence: Synthetic peptide"
CALGETYGGGPLYTDKLIF

SEQ ID NO: 12 - protein, 19 aa, Artificial Sequence
  source: /note="Description of Artificial Sequence: Synthetic peptide"
CALGNTYGGGPLYTDKLIF

SEQ ID NO: 13 - protein, 19 aa, Artificial Sequence
  source: /note="Description of Artificial Sequence: Synthetic peptide"
CALGQTYGGGPLYTDKLIF

SEQ ID NO: 14 - protein, 19 aa, Artificial Sequence
  source: /note="Description of Artificial Sequence: Synthetic peptide"
CALGDSFGGGPLYTDKLIF

SEQ ID NO: 15 - protein, 19 aa, Artificial Sequence
  source: /note="Description of Artificial Sequence: Synthetic peptide"
CALGESFGGGPLYTDKLIF

SEQ ID NO: 16 - protein, 19 aa, Artificial Sequence
  source: /note="Description of Artificial Sequence: Synthetic peptide"
CALGNSFGGGPLYTDKLIF

SEQ ID NO: 17 - protein, 19 aa, Artificial Sequence
  source: /note="Description of Artificial Sequence: Synthetic peptide"
CALGQSFGGGPLYTDKLIF

SEQ ID NO: 18 - protein, 19 aa, Artificial Sequence
  source: /note="Description of Artificial Sequence: Synthetic peptide"
CALGDTFGGGPLYTDKLIF

SEQ ID NO: 19 - protein, 19 aa, Artificial Sequence
  source: /note="Description of Artificial Sequence: Synthetic peptide"
CALGETFGGGPLYTDKLIF

SEQ ID NO: 20 - protein, 19 aa, Artificial Sequence
  source: /note="Description of Artificial Sequence: Synthetic peptide"
CALGNTFGGGPLYTDKLIF

SEQ ID NO: 21 - protein, 19 aa, Artificial Sequence
  source: /note="Description of Artificial Sequence: Synthetic peptide"
CALGQTFGGGPLYTDKLIF

SEQ ID NO: 22 - protein, 19 aa, Artificial Sequence
  source: /note="Description of Artificial Sequence: Synthetic peptide"
CALGDSYAGGPLYTDKLIF

SEQ ID NO: 23 - protein, 19 aa, Artificial Sequence
  source: /note="Description of Artificial Sequence: Synthetic peptide"
CALGESYAGGPLYTDKLIF

SEQ ID NO: 24 - protein, 19 aa, Artificial Sequence
  source: /note="Description of Artificial Sequence: Synthetic peptide"
CALGNSYAGGPLYTDKLIF

SEQ ID NO: 25 - protein, 19 aa, Artificial Sequence
  source: /note="Description of Artificial Sequence: Synthetic peptide"
CALGQSYAGGPLYTDKLIF

SEQ ID NO: 26 - protein, 19 aa, Artificial Sequence
  source: /note="Description of Artificial Sequence: Synthetic peptide"
CALGDTYAGGPLYTDKLIF

SEQ ID NO: 27 - protein, 19 aa, Artificial Sequence
  source: /note="Description of Artificial Sequence: Synthetic peptide"
CALGETYAGGPLYTDKLIF

SEQ ID NO: 28 - protein, 19 aa, Artificial Sequence
  source: /note="Description of Artificial Sequence: Synthetic peptide"
CALGNTYAGGPLYTDKLIF

SEQ ID NO: 29 - protein, 19 aa, Artificial Sequence
  source: /note="Description of Artificial Sequence: Synthetic peptide"
CALGQTYAGGPLYTDKLIF

SEQ ID NO: 30 - protein, 19 aa, Artificial Sequence
  source: /note="Description of Artificial Sequence: Synthetic peptide"
CALGDSYGAGPLYTDKLIF

SEQ ID NO: 31 - protein, 19 aa, Artificial Sequence
  source: /note="Description of Artificial Sequence: Synthetic peptide"
CALGESYGAGPLYTDKLIF

SEQ ID NO: 32 - protein, 19 aa, Artificial Sequence
  source: /note="Description of Artificial Sequence: Synthetic peptide"
CALGNSYGAGPLYTDKLIF

SEQ ID NO: 33 - protein, 19 aa, Artificial Sequence
  source: /note="Description of Artificial Sequence: Synthetic peptide"
CALGQSYGAGPLYTDKLIF

SEQ ID NO: 34 - protein, 19 aa, Artificial Sequence
  source: /note="Description of Artificial Sequence: Synthetic peptide"
CALGDTYGAGPLYTDKLIF

SEQ ID NO: 35 - protein, 19 aa, Artificial Sequence
  source: /note="Description of Artificial Sequence: Synthetic peptide"
CALGETYGAGPLYTDKLIF

SEQ ID NO: 36 - protein, 19 aa, Artificial Sequence
  source: /note="Description of Artificial Sequence: Synthetic peptide"
CALGNTYGAGPLYTDKLIF

SEQ ID NO: 37 - protein, 19 aa, Artificial Sequence
  source: /note="Description of Artificial Sequence: Synthetic peptide"
CALGQTYGAGPLYTDKLIF

SEQ ID NO: 38 - protein, 19 aa, Artificial Sequence
  source: /note="Description of Artificial Sequence: Synthetic peptide"
CALGDSYGGAPLYTDKLIF

SEQ ID NO: 39 - protein, 19 aa, Artificial Sequence
  source: /note="Description of Artificial Sequence: Synthetic peptide"
CALGESYGGAPLYTDKLIF

SEQ ID NO: 40 - protein, 19 aa, Artificial Sequence
  source: /note="Description of Artificial Sequence: Synthetic peptide"
CALGNSYGGAPLYTDKLIF

SEQ ID NO: 41 - protein, 19 aa, Artificial Sequence
  source: /note="Description of Artificial Sequence: Synthetic peptide"
CALGQSYGGAPLYTDKLIF

SEQ ID NO: 42 - protein, 19 aa, Artificial Sequence
  source: /note="Description of Artificial Sequence: Synthetic peptide"
CALGDTYGGAPLYTDKLIF

SEQ ID NO: 43 - protein, 19 aa, Artificial Sequence
  source: /note="Description of Artificial Sequence: Synthetic peptide"
CALGETYGGAPLYTDKLIF

SEQ ID NO: 44 - protein, 19 aa, Artificial Sequence
  source: /note="Description of Artificial Sequence: Synthetic peptide"
CALGNTYGGAPLYTDKLIF

SEQ ID NO: 45 - protein, 19 aa, Artificial Sequence
  source: /note="Description of Artificial Sequence: Synthetic peptide"
CALGQTYGGAPLYTDKLIF

SEQ ID NO: 46 - protein, 19 aa, Artificial Sequence
  source: /note="Description of Artificial Sequence: Synthetic peptide"
CALGDSYGGGPIYTDKLIF

SEQ ID NO: 47 - protein, 19 aa, Artificial Sequence
  source: /note="Description of Artificial Sequence: Synthetic peptide"
CALGESYGGGPIYTDKLIF

SEQ ID NO: 48 - protein, 19 aa, Artificial Sequence
  source: /note="Description of Artificial Sequence: Synthetic peptide"
CALGNSYGGGPIYTDKLIF

SEQ ID NO: 49 - protein, 19 aa, Artificial Sequence
  source: /note="Description of Artificial Sequence: Synthetic peptide"
CALGQSYGGGPIYTDKLIF

SEQ ID NO: 50 - protein, 19 aa, Artificial Sequence
  source: /note="Description of Artificial Sequence: Synthetic peptide"
CALGDTYGGGPIYTDKLIF

SEQ ID NO: 51 - protein, 19 aa, Artificial Sequence
  source: /note="Description of Artificial Sequence: Synthetic peptide"
CALGETYGGGPIYTDKLIF

SEQ ID NO: 52 - protein, 19 aa, Artificial Sequence
  source: /note="Description of Artificial Sequence: Synthetic peptide"
CALGNTYGGGPIYTDKLIF

SEQ ID NO: 53 - protein, 19 aa, Artificial Sequence
  source: /note="Description of Artificial Sequence: Synthetic peptide"
CALGQTYGGGPIYTDKLIF

SEQ ID NO: 54 - protein, 19 aa, Artificial Sequence
  source: /note="Description of Artificial Sequence: Synthetic peptide"
CALGDSFGGGPIYTDKLIF

SEQ ID NO: 55 - protein, 19 aa, Artificial Sequence
  source: /note="Description of Artificial Sequence: Synthetic peptide"
CALGESFGGGPIYTDKLIF

SEQ ID NO: 56 - protein, 19 aa, Artificial Sequence
  source: /note="Description of Artificial Sequence: Synthetic peptide"
CALGNSFGGGPIYTDKLIF

SEQ ID NO: 57 - protein, 19 aa, Artificial Sequence
  source: /note="Description of Artificial Sequence: Synthetic peptide"
CALGQSFGGGPIYTDKLIF

SEQ ID NO: 58 - protein, 19 aa, Artificial Sequence
  source: /note="Description of Artificial Sequence: Synthetic peptide"
CALGDSYGGGPLFTDKLIF

SEQ ID NO: 59 - protein, 19 aa, Artificial Sequence
  source: /note="Description of Artificial Sequence: Synthetic peptide"
CALGESYGGGPLFTDKLIF

SEQ ID NO: 60 - protein, 19 aa, Artificial Sequence
  source: /note="Description of Artificial Sequence: Synthetic peptide"
CALGNSYGGGPLFTDKLIF

SEQ ID NO: 61 - protein, 19 aa, Artificial Sequence
  source: /note="Description of Artificial Sequence: Synthetic peptide"
CALGQSYGGGPLFTDKLIF

SEQ ID NO: 62 - protein, 19 aa, Artificial Sequence
  source: /note="Description of Artificial Sequence: Synthetic peptide"
CALGDTYGGGPLFTDKLIF

SEQ ID NO: 63 - protein, 19 aa, Artificial Sequence
  source: /note="Description of Artificial Sequence: Synthetic peptide"
CALGETYGGGPLFTDKLIF

SEQ ID NO: 64 - protein, 19 aa, Artificial Sequence
  source: /note="Description of Artificial Sequence: Synthetic peptide"
CALGNTYGGGPLFTDKLIF

SEQ ID NO: 65 - protein, 19 aa, Artificial Sequence
  source: /note="Description of Artificial Sequence: Synthetic peptide"
CALGQTYGGGPLFTDKLIF

SEQ ID NO: 66 - protein, 19 aa, Artificial Sequence
  source: /note="Description of Artificial Sequence: Synthetic peptide"
CALGDSFGGGPLFTDKLIF

SEQ ID NO: 67 - protein, 19 aa, Artificial Sequence
  source: /note="Description of Artificial Sequence: Synthetic peptide"
CALGESFGGGPLFTDKLIF

SEQ ID NO: 68 - protein, 19 aa, Artificial Sequence
  source: /note="Description of Artificial Sequence: Synthetic peptide"
CALGNSFGGGPLFTDKLIF

SEQ ID NO: 69 - protein, 19 aa, Artificial Sequence
  source: /note="Description of Artificial Sequence: Synthetic peptide"
CALGQSFGGGPLFTDKLIF

SEQ ID NO: 70 - protein, 19 aa, Artificial Sequence
  source: /note="Description of Artificial Sequence: Synthetic peptide"
CALGDSYGGGPIYSDKLIF

SEQ ID NO: 71 - protein, 19 aa, Artificial Sequence
  source: /note="Description of Artificial Sequence: Synthetic peptide"
CALGESYGGGPIYSDKLIF

SEQ ID NO: 72 - protein, 19 aa, Artificial Sequence
  source: /note="Description of Artificial Sequence: Synthetic peptide"
CALGNSYGGGPIYSDKLIF

SEQ ID NO: 73 - protein, 19 aa, Artificial Sequence
  source: /note="Description of Artificial Sequence: Synthetic peptide"
CALGQSYGGGPIYSDKLIF

SEQ ID NO: 74 - protein, 19 aa, Artificial Sequence
  source: /note="Description of Artificial Sequence: Synthetic peptide"
CALGDTYGGGPIYSDKLIF

SEQ ID NO: 75 - protein, 19 aa, Artificial Sequence
  source: /note="Description of Artificial Sequence: Synthetic peptide"
CALGETYGGGPIYSDKLIF

SEQ ID NO: 76 - protein, 19 aa, Artificial Sequence
  source: /note="Description of Artificial Sequence: Synthetic peptide"
CALGNTYGGGPIYSDKLIF

SEQ ID NO: 77 - protein, 19 aa, Artificial Sequence
  source: /note="Description of Artificial Sequence: Synthetic peptide"
CALGQTYGGGPIYSDKLIF

SEQ ID NO: 78 - protein, 19 aa, Artificial Sequence
  source: /note="Description of Artificial Sequence: Synthetic peptide"
CALGDSFGGGPIYSDKLIF

SEQ ID NO: 79 - protein, 19 aa, Artificial Sequence
  source: /note="Description of Artificial Sequence: Synthetic peptide"
CALGESFGGGPIYSDKLIF

SEQ ID NO: 80 - protein, 19 aa, Artificial Sequence
  source: /note="Description of Artificial Sequence: Synthetic peptide"
CALGNSFGGGPIYSDKLIF

SEQ ID NO: 81 - protein, 19 aa, Artificial Sequence
  source: /note="Description of Artificial Sequence: Synthetic peptide"
CALGQSFGGGPIYSDKLIF

SEQ ID NO: 82 - protein, 19 aa, Artificial Sequence
  source: /note="Description of Artificial Sequence: Synthetic peptide"
CALGDSYGGGPLFSDKLIF

SEQ ID NO: 83 - protein, 19 aa, Artificial Sequence
  source: /note="Description of Artificial Sequence: Synthetic peptide"
CALGESYGGGPLFSDKLIF

SEQ ID NO: 84 - protein, 19 aa, Artificial Sequence
  source: /note="Description of Artificial Sequence: Synthetic peptide"
CALGNSYGGGPLFSDKLIF

SEQ ID NO: 85 - protein, 19 aa, Artificial Sequence
  source: /note="Description of Artificial Sequence: Synthetic peptide"
CALGQSYGGGPLFSDKLIF

SEQ ID NO: 86 - protein, 19 aa, Artificial Sequence
  source: /note="Description of Artificial Sequence: Synthetic peptide"
CALGDTYGGGPLFSDKLIF

SEQ ID NO: 87 - protein, 19 aa, Artificial Sequence
  source: /note="Description of Artificial Sequence: Synthetic peptide"
CALGETYGGGPLFSDKLIF

SEQ ID NO: 88 - protein, 19 aa, Artificial Sequence
  source: /note="Description of Artificial Sequence: Synthetic peptide"
CALGNTYGGGPLFSDKLIF

SEQ ID NO: 89 - protein, 19 aa, Artificial Sequence
  source: /note="Description of Artificial Sequence: Synthetic peptide"
CALGQTYGGGPLFSDKLIF

SEQ ID NO: 90 - protein, 19 aa, Artificial Sequence
  source: /note="Description of Artificial Sequence: Synthetic peptide"
CALGDSFGGGPLFSDKLIF

SEQ ID NO: 91 - protein, 19 aa, Artificial Sequence
  source: /note="Description of Artificial Sequence: Synthetic peptide"
CALGESFGGGPLFSDKLIF

SEQ ID NO: 92 - protein, 19 aa, Artificial Sequence
  source: /note="Description of Artificial Sequence: Synthetic peptide"
CALGNSFGGGPLFSDKLIF

SEQ ID NO: 93 - protein, 19 aa, Artificial Sequence
  source: /note="Description of Artificial Sequence: Synthetic peptide"
CALGQSFGGGPLFSDKLIF

SEQ ID NO: 94 - protein, 19 aa, Artificial Sequence
  source: /note="Description of Artificial Sequence: Synthetic peptide"
CALGDSYGGGPIYTEKLIF

SEQ ID NO: 95 - protein, 19 aa, Artificial Sequence
  source: /note="Description of Artificial Sequence: Synthetic peptide"
CALGESYGGGPIYTEKLIF

SEQ ID NO: 96 - protein, 19 aa, Artificial Sequence
  source: /note="Description of Artificial Sequence: Synthetic peptide"
CALGNSYGGGPIYTEKLIF

SEQ ID NO: 97 - protein, 19 aa, Artificial Sequence
  source: /note="Description of Artificial Sequence: Synthetic peptide"
CALGQSYGGGPIYTEKLIF

SEQ ID NO: 98 - protein, 19 aa, Artificial Sequence
  source: /note="Description of Artificial Sequence: Synthetic peptide"
CALGDTYGGGPIYTEKLIF

SEQ ID NO: 99 - protein, 19 aa, Artificial Sequence
  source: /note="Description of Artificial Sequence: Synthetic peptide"
CALGETYGGGPIYTEKLIF

SEQ ID NO: 100 - protein, 19 aa, Artificial Sequence
  source: /note="Description of Artificial Sequence: Synthetic peptide"
CALGNTYGGGPIYTEKLIF

SEQ ID NO: 101 - protein, 19 aa, Artificial Sequence
  source: /note="Description of Artificial Sequence: Synthetic peptide"
CALGQTYGGGPIYTEKLIF

SEQ ID NO: 102 - protein, 19 aa, Artificial Sequence
  source: /note="Description of Artificial Sequence: Synthetic peptide"
CALGDSFGGGPIYTEKLIF

SEQ ID NO: 103 - protein, 19 aa, Artificial Sequence
  source: /note="Description of Artificial Sequence: Synthetic peptide"
CALGESFGGGPIYTEKLIF

SEQ ID NO: 104 - protein, 19 aa, Artificial Sequence
  source: /note="Description of Artificial Sequence: Synthetic peptide"
CALGNSFGGGPIYTEKLIF

SEQ ID NO: 105 - protein, 19 aa, Artificial Sequence
  source: /note="Description of Artificial Sequence: Synthetic peptide"
CALGQSFGGGPIYTEKLIF

SEQ ID NO: 106 - protein, 19 aa, Artificial Sequence
  source: /note="Description of Artificial Sequence: Synthetic peptide"
CALGDSYGGGPLFTEKLIF

SEQ ID NO: 107 - protein, 19 aa, Artificial Sequence
  source: /note="Description of Artificial Sequence: Synthetic peptide"
CALGESYGGGPLFTEKLIF

SEQ ID NO: 108 - protein, 19 aa, Artificial Sequence
  source: /note="Description of Artificial Sequence: Synthetic peptide"
CALGNSYGGGPLFTEKLIF

SEQ ID NO: 109 - protein, 19 aa, Artificial Sequence
  source: /note="Description of Artificial Sequence: Synthetic peptide"
CALGQSYGGGPLFTEKLIF

SEQ ID NO: 110 - protein, 19 aa, Artificial Sequence
  source: /note="Description of Artificial Sequence: Synthetic peptide"
CALGDTYGGGPLFTEKLIF

SEQ ID NO: 111 - protein, 19 aa, Artificial Sequence
  source: /note="Description of Artificial Sequence: Synthetic peptide"
CALGETYGGGPLFTEKLIF

SEQ ID NO: 112 - protein, 19 aa, Artificial Sequence
  source: /note="Description of Artificial Sequence: Synthetic peptide"
CALGNTYGGGPLFTEKLIF

SEQ ID NO: 113 - protein, 19 aa, Artificial Sequence
  source: /note="Description of Artificial Sequence: Synthetic peptide"
CALGQTYGGGPLFTEKLIF

SEQ ID NO: 114 - protein, 19 aa, Artificial Sequence
  source: /note="Description of Artificial Sequence: Synthetic peptide"
CALGDSFGGGPLFTEKLIF

SEQ ID NO: 115 - protein, 19 aa, Artificial Sequence
  source: /note="Description of Artificial Sequence: Synthetic peptide"
CALGESFGGGPLFTEKLIF

SEQ ID NO: 116 - protein, 19 aa, Artificial Sequence
  source: /note="Description of Artificial Sequence: Synthetic peptide"
CALGNSFGGGPLFTEKLIF

SEQ ID NO: 117 - protein, 19 aa, Artificial Sequence
  source: /note="Description of Artificial Sequence: Synthetic peptide"
CALGQSFGGGPLFTEKLIF

SEQ ID NO: 118 - protein, 19 aa, Artificial Sequence
  source: /note="Description of Artificial Sequence: Synthetic peptide"
CALGDSYGGGPIYTNKLIF

SEQ ID NO: 119 - protein, 19 aa, Artificial Sequence
  source: /note="Description of Artificial Sequence: Synthetic peptide"
CALGESYGGGPIYTNKLIF

SEQ ID NO: 120 - protein, 19 aa, Artificial Sequence
  source: /note="Description of Artificial Sequence: Synthetic peptide"
CALGNSYGGGPIYTNKLIF

SEQ ID NO: 121 - protein, 19 aa, Artificial Sequence
  source: /note="Description of Artificial Sequence: Synthetic peptide"
CALGQSYGGGPIYTNKLIF

SEQ ID NO: 122 - protein, 19 aa, Artificial Sequence
  source: /note="Description of Artificial Sequence: Synthetic peptide"
CALGDTYGGGPIYTNKLIF

SEQ ID NO: 123 - protein, 19 aa, Artificial Sequence
  source: /note="Description of Artificial Sequence: Synthetic peptide"
CALGETYGGGPIYTNKLIF

SEQ ID NO: 124 - protein, 19 aa, Artificial Sequence
  source: /note="Description of Artificial Sequence: Synthetic peptide"
CALGNTYGGGPIYTNKLIF

SEQ ID NO: 125 - protein, 19 aa, Artificial Sequence
  source: /note="Description of Artificial Sequence: Synthetic peptide"
CALGQTYGGGPIYTNKLIF

SEQ ID NO: 126 - protein, 19 aa, Artificial Sequence
  source: /note="Description of Artificial Sequence: Synthetic peptide"
CALGDSFGGGPIYTNKLIF

SEQ ID NO: 127 - protein, 19 aa, Artificial Sequence
  source: /note="Description of Artificial Sequence: Synthetic peptide"
CALGESFGGGPIYTNKLIF

SEQ ID NO: 128 - protein, 19 aa, Artificial Sequence
  source: /note="Description of Artificial Sequence: Synthetic peptide"
CALGNSFGGGPIYTNKLIF

SEQ ID NO: 129 - protein, 19 aa, Artificial Sequence
  source: /note="Description of Artificial Sequence: Synthetic peptide"
CALGQSFGGGPIYTNKLIF

SEQ ID NO: 130 - protein, 19 aa, Artificial Sequence
  source: /note="Description of Artificial Sequence: Synthetic peptide"
CALGDSYGGGPLFTNKLIF

SEQ ID NO: 131 - protein, 19 aa, Artificial Sequence
  source: /note="Description of Artificial Sequence: Synthetic peptide"
CALGESYGGGPLFTNKLIF

SEQ ID NO: 132 - protein, 19 aa, Artificial Sequence
  source: /note="Description of Artificial Sequence: Synthetic peptide"
CALGNSYGGGPLFTNKLIF

SEQ ID NO: 133 - protein, 19 aa, Artificial Sequence
  source: /note="Description of Artificial Sequence: Synthetic peptide"
CALGQSYGGGPLFTNKLIF

SEQ ID NO: 134 - protein, 19 aa, Artificial Sequence
  source: /note="Description of Artificial Sequence: Synthetic peptide"
CALGDTYGGGPLFTNKLIF

SEQ ID NO: 135 - protein, 19 aa, Artificial Sequence
  source: /note="Description of Artificial Sequence: Synthetic peptide"
CALGETYGGGPLFTNKLIF

SEQ ID NO: 136 - protein, 19 aa, Artificial Sequence
  source: /note="Description of Artificial Sequence: Synthetic peptide"
CALGNTYGGGPLFTNKLIF

SEQ ID NO: 137 - protein, 19 aa, Artificial Sequence
  source: /note="Description of Artificial Sequence: Synthetic peptide"
CALGQTYGGGPLFTNKLIF

SEQ ID NO: 138 - protein, 19 aa, Artificial Sequence
  source: /note="Description of Artificial Sequence: Synthetic peptide"
CALGDSFGGGPLFTNKLIF

SEQ ID NO: 139 - protein, 19 aa, Artificial Sequence
  source: /note="Description of Artificial Sequence: Synthetic peptide"
CALGESFGGGPLFTNKLIF

SEQ ID NO: 140 - protein, 19 aa, Artificial Sequence
  source: /note="Description of Artificial Sequence: Synthetic peptide"
CALGNSFGGGPLFTNKLIF

SEQ ID NO: 141 - protein, 19 aa, Artificial Sequence
  source: /note="Description of Artificial Sequence: Synthetic peptide"
CALGQSFGGGPLFTNKLIF

SEQ ID NO: 142 - protein, 19 aa, Artificial Sequence
  source: /note="Description of Artificial Sequence: Synthetic peptide"
CALGDSYGGGPIYSEKLIF

SEQ ID NO: 143 - protein, 19 aa, Artificial Sequence
  source: /note="Description of Artificial Sequence: Synthetic peptide"
CALGESYGGGPIYSEKLIF

SEQ ID NO: 144 - protein, 19 aa, Artificial Sequence
  source: /note="Description of Artificial Sequence: Synthetic peptide"
CALGNSYGGGPIYSEKLIF

SEQ ID NO: 145 - protein, 19 aa, Artificial Sequence
  source: /note="Description of Artificial Sequence: Synthetic peptide"
CALGQSYGGGPIYSEKLIF

SEQ ID NO: 146 - protein, 19 aa, Artificial Sequence
  source: /note="Description of Artificial Sequence: Synthetic peptide"
CALGDTYGGGPIYSEKLIF

SEQ ID NO: 147 - protein, 19 aa, Artificial Sequence
  source: /note="Description of Artificial Sequence: Synthetic peptide"
CALGETYGGGPIYSEKLIF

SEQ ID NO: 148 - protein, 19 aa, Artificial Sequence
  source: /note="Description of Artificial Sequence: Synthetic peptide"
CALGNTYGGGPIYSEKLIF

SEQ ID NO: 149 - protein, 19 aa, Artificial Sequence
  source: /note="Description of Artificial Sequence: Synthetic peptide"
CALGQTYGGGPIYSEKLIF

SEQ ID NO: 150 - protein, 19 aa, Artificial Sequence
  source: /note="Description of Artificial Sequence: Synthetic peptide"
CALGDSFGGGPIYSEKLIF

SEQ ID NO: 151 - protein, 19 aa, Artificial Sequence
  source: /note="Description of Artificial Sequence: Synthetic peptide"
CALGESFGGGPIYSEKLIF

SEQ ID NO: 152 - protein, 19 aa, Artificial Sequence
  source: /note="Description of Artificial Sequence: Synthetic peptide"
CALGNSFGGGPIYSEKLIF

SEQ ID NO: 153 - protein, 19 aa, Artificial Sequence
  source: /note="Description of Artificial Sequence: Synthetic peptide"
CALGQSFGGGPIYSEKLIF

SEQ ID NO: 154 - protein, 19 aa, Artificial Sequence
  source: /note="Description of Artificial Sequence: Synthetic peptide"
CALGDSYGGGPLFSEKLIF

SEQ ID NO: 155 - protein, 19 aa, Artificial Sequence
  source: /note="Description of Artificial Sequence: Synthetic peptide"
CALGESYGGGPLFSEKLIF

SEQ ID NO: 156 - protein, 19 aa, Artificial Sequence
  source: /note="Description of Artificial Sequence: Synthetic peptide"
CALGNSYGGGPLFSEKLIF

SEQ ID NO: 157 - protein, 19 aa, Artificial Sequence
  source: /note="Description of Artificial Sequence: Synthetic peptide"
CALGQSYGGGPLFSEKLIF

SEQ ID NO: 158 - protein, 19 aa, Artificial Sequence
  source: /note="Description of Artificial Sequence: Synthetic peptide"
CALGDTYGGGPLFSEKLIF

SEQ ID NO: 159 - protein, 19 aa, Artificial Sequence
  source: /note="Description of Artificial Sequence: Synthetic peptide"
CALGETYGGGPLFSEKLIF

SEQ ID NO: 160 - protein, 19 aa, Artificial Sequence
  source: /note="Description of Artificial Sequence: Synthetic peptide"
CALGNTYGGGPLFSEKLIF

SEQ ID NO: 161 - protein, 19 aa, Artificial Sequence
  source: /note="Description of Artificial Sequence: Synthetic peptide"
CALGQTYGGGPLFSEKLIF

SEQ ID NO: 162 - protein, 19 aa, Artificial Sequence
  source: /note="Description of Artificial Sequence: Synthetic peptide"
CALGDSFGGGPLFSEKLIF

SEQ ID NO: 163 - protein, 19 aa, Artificial Sequence
  source: /note="Description of Artificial Sequence: Synthetic peptide"
CALGESFGGGPLFSEKLIF

SEQ ID NO: 164 - protein, 19 aa, Artificial Sequence
  source: /note="Description of Artificial Sequence: Synthetic peptide"
CALGNSFGGGPLFSEKLIF

SEQ ID NO: 165 - protein, 19 aa, Artificial Sequence
  source: /note="Description of Artificial Sequence: Synthetic peptide"
CALGQSFGGGPLFSEKLIF

SEQ ID NO: 166 - protein, 19 aa, Artificial Sequence
  source: /note="Description of Artificial Sequence: Synthetic peptide"
CALGDSYGGGPIYSNKLIF

SEQ ID NO: 167 - protein, 19 aa, Artificial Sequence
  source: /note="Description of Artificial Sequence: Synthetic peptide"
CALGESYGGGPIYSNKLIF

SEQ ID NO: 168 - protein, 19 aa, Artificial Sequence
  source: /note="Description of Artificial Sequence: Synthetic peptide"
CALGNSYGGGPIYSNKLIF

SEQ ID NO: 169 - protein, 19 aa, Artificial Sequence
  source: /note="Description of Artificial Sequence: Synthetic peptide"
CALGQSYGGGPIYSNKLIF

SEQ ID NO: 170 - protein, 19 aa, Artificial Sequence
  source: /note="Description of Artificial Sequence: Synthetic peptide"
CALGDTYGGGPIYSNKLIF

SEQ ID NO: 171 - protein, 19 aa, Artificial Sequence
  source: /note="Description of Artificial Sequence: Synthetic peptide"
CALGETYGGGPIYSNKLIF

SEQ ID NO: 172 - protein, 19 aa, Artificial Sequence
  source: /note="Description of Artificial Sequence: Synthetic peptide"
CALGNTYGGGPIYSNKLIF

SEQ ID NO: 173 - protein, 19 aa, Artificial Sequence
  source: /note="Description of Artificial Sequence: Synthetic peptide"
CALGQTYGGGPIYSNKLIF

SEQ ID NO: 174 - protein, 19 aa, Artificial Sequence
  source: /note="Description of Artificial Sequence: Synthetic peptide"
CALGDSFGGGPIYSNKLIF

SEQ ID NO: 175 - protein, 19 aa, Artificial Sequence
  source: /note="Description of Artificial Sequence: Synthetic peptide"
CALGESFGGGPIYSNKLIF

SEQ ID NO: 176 - protein, 19 aa, Artificial Sequence
  source: /note="Description of Artificial Sequence: Synthetic peptide"
CALGNSFGGGPIYSNKLIF

SEQ ID NO: 177 - protein, 19 aa, Artificial Sequence
  source: /note="Description of Artificial Sequence: Synthetic peptide"
CALGQSFGGGPIYSNKLIF

SEQ ID NO: 178 - protein, 19 aa, Artificial Sequence
  source: /note="Description of Artificial Sequence: Synthetic peptide"
CALGDSYGGGPLFSNKLIF

SEQ ID NO: 179 - protein, 19 aa, Artificial Sequence
  source: /note="Description of Artificial Sequence: Synthetic peptide"
CALGESYGGGPLFSNKLIF

SEQ ID NO: 180 - protein, 19 aa, Artificial Sequence
  source: /note="Description of Artificial Sequence: Synthetic peptide"
CALGNSYGGGPLFSNKLIF

SEQ ID NO: 181 - protein, 19 aa, Artificial Sequence
  source: /note="Description of Artificial Sequence: Synthetic peptide"
CALGQSYGGGPLFSNKLIF

SEQ ID NO: 182 - protein, 19 aa, Artificial Sequence
  source: /note="Description of Artificial Sequence: Synthetic peptide"
CALGDTYGGGPLFSNKLIF

SEQ ID NO: 183 - protein, 19 aa, Artificial Sequence
  source: /note="Description of Artificial Sequence: Synthetic peptide"
CALGETYGGGPLFSNKLIF

SEQ ID NO: 184 - protein, 19 aa, Artificial Sequence
  source: /note="Description of Artificial Sequence: Synthetic peptide"
CALGNTYGGGPLFSNKLIF

SEQ ID NO: 185 - protein, 19 aa, Artificial Sequence
  source: /note="Description of Artificial Sequence: Synthetic peptide"
CALGQTYGGGPLFSNKLIF

SEQ ID NO: 186 - protein, 19 aa, Artificial Sequence
  source: /note="Description of Artificial Sequence: Synthetic peptide"
CALGDSFGGGPLFSNKLIF

SEQ ID NO: 187 - protein, 19 aa, Artificial Sequence
  source: /note="Description of Artificial Sequence: Synthetic peptide"
CALGESFGGGPLFSNKLIF

SEQ ID NO: 188 - protein, 19 aa, Artificial Sequence
  source: /note="Description of Artificial Sequence: Synthetic peptide"
CALGNSFGGGPLFSNKLIF

SEQ ID NO: 189 - protein, 19 aa, Artificial Sequence
  source: /note="Description of Artificial Sequence: Synthetic peptide"
CALGQSFGGGPLFSNKLIF

SEQ ID NO: 190 - protein, 19 aa, Artificial Sequence
  source: /note="Description of Artificial Sequence: Synthetic peptide"
CALGDSYGGGPIYTDRLIF

SEQ ID NO: 191 - protein, 19 aa, Artificial Sequence
  source: /note="Description of Artificial Sequence: Synthetic peptide"
CALGESYGGGPIYTDRLIF

SEQ ID NO: 192 - protein, 19 aa, Artificial Sequence
  source: /note="Description of Artificial Sequence: Synthetic peptide"
CALGNSYGGGPIYTDRLIF

SEQ ID NO: 193 - protein, 19 aa, Artificial Sequence
  source: /note="Description of Artificial Sequence: Synthetic peptide"
CALGQSYGGGPIYTDRLIF

SEQ ID NO: 194 - protein, 19 aa, Artificial Sequence
  source: /note="Description of Artificial Sequence: Synthetic peptide"
CALGDTYGGGPIYTDRLIF

SEQ ID NO: 195 - protein, 19 aa, Artificial Sequence
  source: /note="Description of Artificial Sequence: Synthetic peptide"
CALGETYGGGPIYTDRLIF

SEQ ID NO: 196 - protein, 19 aa, Artificial Sequence
  source: /note="Description of Artificial Sequence: Synthetic peptide"
CALGNTYGGGPIYTDRLIF

SEQ ID NO: 197 - protein, 19 aa, Artificial Sequence
  source: /note="Description of Artificial Sequence: Synthetic peptide"
CALGQTYGGGPIYTDRLIF

SEQ ID NO: 198 - protein, 19 aa, Artificial Sequence
  source: /note="Description of Artificial Sequence: Synthetic peptide"
CALGDSFGGGPIYTDRLIF

SEQ ID NO: 199 - protein, 19 aa, Artificial Sequence
  source: /note="Description of Artificial Sequence: Synthetic peptide"
CALGESFGGGPIYTDRLIF

SEQ ID NO: 200 - protein, 19 aa, Artificial Sequence
  source: /note="Description of Artificial Sequence: Synthetic peptide"
CALGNSFGGGPIYTDRLIF

SEQ ID NO: 201 - protein, 19 aa, Artificial Sequence
  source: /note="Description of Artificial Sequence: Synthetic peptide"
CALGQSFGGGPIYTDRLIF

SEQ ID NO: 202 - protein, 19 aa, Artificial Sequence
  source: /note="Description of Artificial Sequence: Synthetic peptide"
CALGDSYGGGPLFTDRLIF

SEQ ID NO: 203 - protein, 19 aa, Artificial Sequence
  source: /note="Description of Artificial Sequence: Synthetic peptide"
CALGESYGGGPLFTDRLIF

SEQ ID NO: 204 - protein, 19 aa, Artificial Sequence
  source: /note="Description of Artificial Sequence: Synthetic peptide"
CALGNSYGGGPLFTDRLIF

SEQ ID NO: 205 - protein, 19 aa, Artificial Sequence
  source: /note="Description of Artificial Sequence: Synthetic peptide"
CALGQSYGGGPLFTDRLIF

SEQ ID NO: 206 - protein, 19 aa, Artificial Sequence
  source: /note="Description of Artificial Sequence: Synthetic peptide"
CALGDTYGGGPLFTDRLIF

SEQ ID NO: 207 - protein, 19 aa, Artificial Sequence
  source: /note="Description of Artificial Sequence: Synthetic peptide"
CALGETYGGGPLFTDRLIF

SEQ ID NO: 208 - protein, 19 aa, Artificial Sequence
  source: /note="Description of Artificial Sequence: Synthetic peptide"
CALGNTYGGGPLFTDRLIF

SEQ ID NO: 209 - protein, 19 aa, Artificial Sequence
  source: /note="Description of Artificial Sequence: Synthetic peptide"
CALGQTYGGGPLFTDRLIF

SEQ ID NO: 210 - protein, 19 aa, Artificial Sequence
  source: /note="Description of Artificial Sequence: Synthetic peptide"
CALGDSFGGGPLFTDRLIF

SEQ ID NO: 211 - protein, 19 aa, Artificial Sequence
  source: /note="Description of Artificial Sequence: Synthetic peptide"
CALGESFGGGPLFTDRLIF

SEQ ID NO: 212 - protein, 19 aa, Artificial Sequence
  source: /note="Description of Artificial Sequence: Synthetic peptide"
CALGNSFGGGPLFTDRLIF

SEQ ID NO: 213 - protein, 19 aa, Artificial Sequence
  source: /note="Description of Artificial Sequence: Synthetic peptide"
CALGQSFGGGPLFTDRLIF

SEQ ID NO: 214 - protein, 19 aa, Artificial Sequence
  source: /note="Description of Artificial Sequence: Synthetic peptide"
CALGDSYGGGPIYSDRLIF

SEQ ID NO: 215 - protein, 19 aa, Artificial Sequence
  source: /note="Description of Artificial Sequence: Synthetic peptide"
CALGESYGGGPIYSDRLIF

SEQ ID NO: 216 - protein, 19 aa, Artificial Sequence
  source: /note="Description of Artificial Sequence: Synthetic peptide"
CALGNSYGGGPIYSDRLIF

SEQ ID NO: 217 - protein, 19 aa, Artificial Sequence
  source: /note="Description of Artificial Sequence: Synthetic peptide"
CALGQSYGGGPIYSDRLIF

SEQ ID NO: 218 - protein, 19 aa, Artificial Sequence
  source: /note="Description of Artificial Sequence: Synthetic peptide"
CALGDTYGGGPIYSDRLIF

SEQ ID NO: 219 - protein, 19 aa, Artificial Sequence
  source: /note="Description of Artificial Sequence: Synthetic peptide"
CALGETYGGGPIYSDRLIF

SEQ ID NO: 220 - protein, 19 aa, Artificial Sequence
  source: /note="Description of Artificial Sequence: Synthetic peptide"
CALGNTYGGGPIYSDRLIF

SEQ ID NO: 221 - protein, 19 aa, Artificial Sequence
  source: /note="Description of Artificial Sequence: Synthetic peptide"
CALGQTYGGGPIYSDRLIF

SEQ ID NO: 222 - protein, 19 aa, Artificial Sequence
  source: /note="Description of Artificial Sequence: Synthetic peptide"
CALGDSFGGGPIYSDRLIF

SEQ ID NO: 223 - protein, 19 aa, Artificial Sequence
  source: /note="Description of Artificial Sequence: Synthetic peptide"
CALGESFGGGPIYSDRLIF

SEQ ID NO: 224 - protein, 19 aa, Artificial Sequence
  source: /note="Description of Artificial Sequence: Synthetic peptide"
CALGNSFGGGPIYSDRLIF

SEQ ID NO: 225 - protein, 19 aa, Artificial Sequence
  source: /note="Description of Artificial Sequence: Synthetic peptide"
CALGQSFGGGPIYSDRLIF

SEQ ID NO: 226 - protein, 19 aa, Artificial Sequence
  source: /note="Description of Artificial Sequence: Synthetic peptide"
CALGDSYGGGPLFSDRLIF

SEQ ID NO: 227 - protein, 19 aa, Artificial Sequence
  source: /note="Description of Artificial Sequence: Synthetic peptide"
CALGESYGGGPLFSDRLIF

SEQ ID NO: 228 - protein, 19 aa, Artificial Sequence
  source: /note="Description of Artificial Sequence: Synthetic peptide"
CALGNSYGGGPLFSDRLIF

SEQ ID NO: 229 - protein, 19 aa, Artificial Sequence
  source: /note="Description of Artificial Sequence: Synthetic peptide"
CALGQSYGGGPLFSDRLIF

SEQ ID NO: 230 - protein, 19 aa, Artificial Sequence
  source: /note="Description of Artificial Sequence: Synthetic peptide"
CALGDTYGGGPLFSDRLIF

SEQ ID NO: 231 - protein, 19 aa, Artificial Sequence
  source: /note="Description of Artificial Sequence: Synthetic peptide"
CALGETYGGGPLFSDRLIF

SEQ ID NO: 232 - protein, 19 aa, Artificial Sequence
  source: /note="Description of Artificial Sequence: Synthetic peptide"
CALGNTYGGGPLFSDRLIF

SEQ ID NO: 233 - protein, 19 aa, Artificial Sequence
  source: /note="Description of Artificial Sequence: Synthetic peptide"
CALGQTYGGGPLFSDRLIF

SEQ ID NO: 234 - protein, 19 aa, Artificial Sequence
  source: /note="Description of Artificial Sequence: Synthetic peptide"
CALGDSFGGGPLFSDRLIF

SEQ ID NO: 235 - protein, 19 aa, Artificial Sequence
  source: /note="Description of Artificial Sequence: Synthetic peptide"
CALGESFGGGPLFSDRLIF

SEQ ID NO: 236 - protein, 19 aa, Artificial Sequence
  source: /note="Description of Artificial Sequence: Synthetic peptide"
CALGNSFGGGPLFSDRLIF

SEQ ID NO: 237 - protein, 19 aa, Artificial Sequence
  source: /note="Description of Artificial Sequence: Synthetic peptide"
CALGQSFGGGPLFSDRLIF

SEQ ID NO: 238 - protein, 15 aa, Artificial Sequence
  source: /note="Description of Artificial Sequence: Synthetic peptide"
CATWDRPEIYYKKLF

SEQ ID NO: 239 - protein, 15 aa, Artificial Sequence
  source: /note="Description of Artificial Sequence: Synthetic peptide"
CATWERPEIYYKKLF

SEQ ID NO: 240 - protein, 15 aa, Artificial Sequence
  source: /note="Description of Artificial Sequence: Synthetic peptide"
CATWNRPEIYYKKLF

SEQ ID NO: 241 - protein, 15 aa, Artificial Sequence
  source: /note="Description of Artificial Sequence: Synthetic peptide"
CATWQRPEIYYKKLF

SEQ ID NO: 242 - protein, 15 aa, Artificial Sequence
  source: /note="Description of Artificial Sequence: Synthetic peptide"
CATWDKPEIYYKKLF

SEQ ID NO: 243 - protein, 15 aa, Artificial Sequence
  source: /note="Description of Artificial Sequence: Synthetic peptide"
CATWEKPEIYYKKLF

SEQ ID NO: 244 - protein, 15 aa, Artificial Sequence
  source: /note="Description of Artificial Sequence: Synthetic peptide"
CATWNKPEIYYKKLF

SEQ ID NO: 245 - protein, 15 aa, Artificial Sequence
  source: /note="Description of Artificial Sequence: Synthetic peptide"
CATWQKPEIYYKKLF

SEQ ID NO: 246 - protein, 15 aa, Artificial Sequence
  source: /note="Description of Artificial Sequence: Synthetic peptide"
CATWDRPDIYYKKLF

SEQ ID NO: 247 - protein, 15 aa, Artificial Sequence
  source: /note="Description of Artificial Sequence: Synthetic peptide"
CATWERPDIYYKKLF

SEQ ID NO: 248 - protein, 15 aa, Artificial Sequence
  source: /note="Description of Artificial Sequence: Synthetic peptide"
CATWNRPDIYYKKLF

SEQ ID NO: 249 - protein, 15 aa, Artificial Sequence
  source: /note="Description of Artificial Sequence: Synthetic peptide"
CATWQRPDIYYKKLF

SEQ ID NO: 250 - protein, 15 aa, Artificial Sequence
  source: /note="Description of Artificial Sequence: Synthetic peptide"
CATWDKPDIYYKKLF

SEQ ID NO: 251 - protein, 15 aa, Artificial Sequence
  source: /note="Description of Artificial Sequence: Synthetic peptide"
CATWEKPDIYYKKLF

SEQ ID NO: 252 - protein, 15 aa, Artificial Sequence
  source: /note="Description of Artificial Sequence: Synthetic peptide"
CATWNKPDIYYKKLF

SEQ ID NO: 253 - protein, 15 aa, Artificial Sequence
  source: /note="Description of Artificial Sequence: Synthetic peptide"
CATWQKPDIYYKKLF

SEQ ID NO: 254 - protein, 15 aa, Artificial Sequence
  source: /note="Description of Artificial Sequence: Synthetic peptide"
CATWDRPNIYYKKLF

SEQ ID NO: 255 - protein, 15 aa, Artificial Sequence
  source: /note="Description of Artificial Sequence: Synthetic peptide"
CATWERPNIYYKKLF

SEQ ID NO: 256 - protein, 15 aa, Artificial Sequence
  source: /note="Description of Artificial Sequence: Synthetic peptide"
CATWNRPNIYYKKLF

SEQ ID NO: 257 - protein, 15 aa, Artificial Sequence
  source: /note="Description of Artificial Sequence: Synthetic peptide"
CATWQRPNIYYKKLF

SEQ ID NO: 258 - protein, 15 aa, Artificial Sequence
  source: /note="Description of Artificial Sequence: Synthetic peptide"
CATWDKPNIYYKKLF

SEQ ID NO: 259 - protein, 15 aa, Artificial Sequence
  source: /note="Description of Artificial Sequence: Synthetic peptide"
CATWEKPNIYYKKLF

SEQ ID NO: 260 - protein, 15 aa, Artificial Sequence
  source: /note="Description of Artificial Sequence: Synthetic peptide"
CATWNKPNIYYKKLF

SEQ ID NO: 261 - protein, 15 aa, Artificial Sequence
  source: /note="Description of Artificial Sequence: Synthetic peptide"
CATWQKPNIYYKKLF

SEQ ID NO: 262 - protein, 15 aa, Artificial Sequence
  source: /note="Description of Artificial Sequence: Synthetic peptide"
CATWDRPQIYYKKLF

SEQ ID NO: 263 - protein, 15 aa, Artificial Sequence
  source: /note="Description of Artificial Sequence: Synthetic peptide"
CATWERPQIYYKKLF

SEQ ID NO: 264 - protein, 15 aa, Artificial Sequence
  source: /note="Description of Artificial Sequence: Synthetic peptide"
CATWNRPQIYYKKLF

SEQ ID NO: 265 - protein, 15 aa, Artificial Sequence
  source: /note="Description of Artificial Sequence: Synthetic peptide"
CATWQRPQIYYKKLF

SEQ ID NO: 266 - protein, 15 aa, Artificial Sequence
  source: /note="Description of Artificial Sequence: Synthetic peptide"
CATWDKPQIYYKKLF

SEQ ID NO: 267 - protein, 15 aa, Artificial Sequence
  source: /note="Description of Artificial Sequence: Synthetic peptide"
CATWEKPQIYYKKLF

SEQ ID NO: 268 - protein, 15 aa, Artificial Sequence
  source: /note="Description of Artificial Sequence: Synthetic peptide"
CATWNKPQIYYKKLF

SEQ ID NO: 269 - protein, 15 aa, Artificial Sequence
  source: /note="Description of Artificial Sequence: Synthetic peptide"
CATWQKPQIYYKKLF

SEQ ID NO: 270 - protein, 15 aa, Artificial Sequence
  source: /note="Description of Artificial Sequence: Synthetic peptide"
CATWDRPELYYKKLF

SEQ ID NO: 271 - protein, 15 aa, Artificial Sequence
  source: /note="Description of Artificial Sequence: Synthetic peptide"
CATWERPELYYKKLF

SEQ ID NO: 272 - protein, 15 aa, Artificial Sequence
  source: /note="Description of Artificial Sequence: Synthetic peptide"
CATWNRPELYYKKLF

SEQ ID NO: 273 - protein, 15 aa, Artificial Sequence
  source: /note="Description of Artificial Sequence: Synthetic peptide"
CATWQRPELYYKKLF

SEQ ID NO: 274 - protein, 15 aa, Artificial Sequence
  source: /note="Description of Artificial Sequence: Synthetic peptide"
CATWDKPELYYKKLF

SEQ ID NO: 275 - protein, 15 aa, Artificial Sequence
  source: /note="Description of Artificial Sequence: Synthetic peptide"
CATWEKPELYYKKLF

SEQ ID NO: 276 - protein, 15 aa, Artificial Sequence
  source: /note="Description of Artificial Sequence: Synthetic peptide"
CATWNKPELYYKKLF

SEQ ID NO: 277 - protein, 15 aa, Artificial Sequence
  source: /note="Description of Artificial Sequence: Synthetic peptide"
CATWQKPELYYKKLF

SEQ ID NO: 278 - protein, 15 aa, Artificial Sequence
  source: /note="Description of Artificial Sequence: Synthetic peptide"
CATWDRPDLYYKKLF

SEQ ID NO: 279 - protein, 15 aa, Artificial Sequence
  source: /note="Description of Artificial Sequence: Synthetic peptide"
CATWERPDLYYKKLF

SEQ ID NO: 280 - protein, 15 aa, Artificial Sequence
  source: /note="Description of Artificial Sequence: Synthetic peptide"
CATWNRPDLYYKKLF

SEQ ID NO: 281 - protein, 15 aa, Artificial Sequence
  source: /note="Description of Artificial Sequence: Synthetic peptide"
CATWQRPDLYYKKLF

SEQ ID NO: 282 - protein, 15 aa, Artificial Sequence
  source: /note="Description of Artificial Sequence: Synthetic peptide"
CATWDKPDLYYKKLF

SEQ ID NO: 283 - protein, 15 aa, Artificial Sequence
  source: /note="Description of Artificial Sequence: Synthetic peptide"
CATWEKPDLYYKKLF

SEQ ID NO: 284 - protein, 15 aa, Artificial Sequence
  source: /note="Description of Artificial Sequence: Synthetic peptide"
CATWNKPDLYYKKLF

SEQ ID NO: 285 - protein, 15 aa, Artificial Sequence
  source: /note="Description of Artificial Sequence: Synthetic peptide"
CATWQKPDLYYKKLF

SEQ ID NO: 286 - protein, 15 aa, Artificial Sequence
  source: /note="Description of Artificial Sequence: Synthetic peptide"
CATWDRPNLYYKKLF

SEQ ID NO: 287 - protein, 15 aa, Artificial Sequence
  source: /note="Description of Artificial Sequence: Synthetic peptide"
CATWERPNLYYKKLF

SEQ ID NO: 288 - protein, 15 aa, Artificial Sequence
  source: /note="Description of Artificial Sequence: Synthetic peptide"
CATWNRPNLYYKKLF

SEQ ID NO: 289 - protein, 15 aa, Artificial Sequence
  source: /note="Description of Artificial Sequence: Synthetic peptide"
CATWQRPNLYYKKLF

SEQ ID NO: 290 - protein, 15 aa, Artificial Sequence
  source: /note="Description of Artificial Sequence: Synthetic peptide"
CATWDKPNLYYKKLF

SEQ ID NO: 291 - protein, 15 aa, Artificial Sequence
  source: /note="Description of Artificial Sequence: Synthetic peptide"
CATWEKPNLYYKKLF

SEQ ID NO: 292 - protein, 15 aa, Artificial Sequence
  source: /note="Description of Artificial Sequence: Synthetic peptide"
CATWNKPNLYYKKLF

SEQ ID NO: 293 - protein, 15 aa, Artificial Sequence
  source: /note="Description of Artificial Sequence: Synthetic peptide"
CATWQKPNLYYKKLF

SEQ ID NO: 294 - protein, 15 aa, Artificial Sequence
  source: /note="Description of Artificial Sequence: Synthetic peptide"
CATWDRPQLYYKKLF

SEQ ID NO: 295 - protein, 15 aa, Artificial Sequence
  source: /note="Description of Artificial Sequence: Synthetic peptide"
CATWERPQLYYKKLF

SEQ ID NO: 296 - protein, 15 aa, Artificial Sequence
  source: /note="Description of Artificial Sequence: Synthetic peptide"
CATWNRPQLYYKKLF

SEQ ID NO: 297 - protein, 15 aa, Artificial Sequence
  source: /note="Description of Artificial Sequence: Synthetic peptide"
CATWQRPQLYYKKLF

SEQ ID NO: 298 - protein, 15 aa, Artificial Sequence
  source: /note="Description of Artificial Sequence: Synthetic peptide"
CATWDKPQLYYKKLF

SEQ ID NO: 299 - protein, 15 aa, Artificial Sequence
  source: /note="Description of Artificial Sequence: Synthetic peptide"
CATWEKPQLYYKKLF

SEQ ID NO: 300 - protein, 15 aa, Artificial Sequence
  source: /note="Description of Artificial Sequence: Synthetic peptide"
CATWNKPQLYYKKLF

SEQ ID NO: 301 - protein, 15 aa, Artificial Sequence
  source: /note="Description of Artificial Sequence: Synthetic peptide"
CATWQKPQLYYKKLF

SEQ ID NO: 302 - protein, 15 aa, Artificial Sequence
  source: /note="Description of Artificial Sequence: Synthetic peptide"
CATWDRPEIFYKKLF

SEQ ID NO: 303 - protein, 15 aa, Artificial Sequence
  source: /note="Description of Artificial Sequence: Synthetic peptide"
CATWERPEIFYKKLF

SEQ ID NO: 304 - protein, 15 aa, Artificial Sequence
  source: /note="Description of Artificial Sequence: Synthetic peptide"
CATWNRPEIFYKKLF

SEQ ID NO: 305 - protein, 15 aa, Artificial Sequence
  source: /note="Description of Artificial Sequence: Synthetic peptide"
CATWQRPEIFYKKLF

SEQ ID NO: 306 - protein, 15 aa, Artificial Sequence
  source: /note="Description of Artificial Sequence: Synthetic peptide"
CATWDKPEIFYKKLF

SEQ ID NO: 307 - protein, 15 aa, Artificial Sequence
  source: /note="Description of Artificial Sequence: Synthetic peptide"
CATWEKPEIFYKKLF

SEQ ID NO: 308 - protein, 15 aa, Artificial Sequence
  source: /note="Description of Artificial Sequence: Synthetic peptide"
CATWNKPEIFYKKLF

SEQ ID NO: 309 - protein, 15 aa, Artificial Sequence
  source: /note="Description of Artificial Sequence: Synthetic peptide"
CATWQKPEIFYKKLF

SEQ ID NO: 310 - protein, 15 aa, Artificial Sequence
  source: /note="Description of Artificial Sequence: Synthetic peptide"
CATWDRPDIFYKKLF

SEQ ID NO: 311 - protein, 15 aa, Artificial Sequence
  source: /note="Description of Artificial Sequence: Synthetic peptide"
CATWERPDIFYKKLF

SEQ ID NO: 312 - protein, 15 aa, Artificial Sequence
  source: /note="Description of Artificial Sequence: Synthetic peptide"
CATWNRPDIFYKKLF

SEQ ID NO: 313 - protein, 15 aa, Artificial Sequence
  source: /note="Description of Artificial Sequence: Synthetic peptide"
CATWQRPDIFYKKLF

SEQ ID NO: 314 - protein, 15 aa, Artificial Sequence
  source: /note="Description of Artificial Sequence: Synthetic peptide"
CATWDKPDIFYKKLF

SEQ ID NO: 315 - protein, 15 aa, Artificial Sequence
  source: /note="Description of Artificial Sequence: Synthetic peptide"
CATWEKPDIFYKKLF

SEQ ID NO: 316 - protein, 15 aa, Artificial Sequence
  source: /note="Description of Artificial Sequence: Synthetic peptide"
CATWNKPDIFYKKLF

SEQ ID NO: 317 - protein, 15 aa, Artificial Sequence
  source: /note="Description of Artificial Sequence: Synthetic peptide"
CATWQKPDIFYKKLF

SEQ ID NO: 318 - protein, 15 aa, Artificial Sequence
  source: /note="Description of Artificial Sequence: Synthetic peptide"
CATWDRPNIFYKKLF

SEQ ID NO: 319 - protein, 15 aa, Artificial Sequence
  source: /note="Description of Artificial Sequence: Synthetic peptide"
CATWERPNIFYKKLF

SEQ ID NO: 320 - protein, 15 aa, Artificial Sequence
  source: /note="Description of Artificial Sequence: Synthetic peptide"
CATWNRPNIFYKKLF

SEQ ID NO: 321 - protein, 15 aa, Artificial Sequence
  source: /note="Description of Artificial Sequence: Synthetic peptide"
CATWQRPNIFYKKLF

SEQ ID NO: 322 - protein, 15 aa, Artificial Sequence
  source: /note="Description of Artificial Sequence: Synthetic peptide"
CATWDKPNIFYKKLF

SEQ ID NO: 323 - protein, 15 aa, Artificial Sequence
  source: /note="Description of Artificial Sequence: Synthetic peptide"
CATWEKPNIFYKKLF

SEQ ID NO: 324 - protein, 15 aa, Artificial Sequence
  source: /note="Description of Artificial Sequence: Synthetic peptide"
CATWNKPNIFYKKLF

SEQ ID NO: 325 - protein, 15 aa, Artificial Sequence
  source: /note="Description of Artificial Sequence: Synthetic peptide"
CATWQKPNIFYKKLF

SEQ ID NO: 326 - protein, 15 aa, Artificial Sequence
  source: /note="Description of Artificial Sequence: Synthetic peptide"
CATWDRPQIFYKKLF

SEQ ID NO: 327 - protein, 15 aa, Artificial Sequence
  source: /note="Description of Artificial Sequence: Synthetic peptide"
CATWERPQIFYKKLF

SEQ ID NO: 328 - protein, 15 aa, Artificial Sequence
  source: /note="Description of Artificial Sequence: Synthetic peptide"
CATWNRPQIFYKKLF

SEQ ID NO: 329 - protein, 15 aa, Artificial Sequence
  source: /note="Description of Artificial Sequence: Synthetic peptide"
CATWQRPQIFYKKLF

SEQ ID NO: 330 - protein, 15 aa, Artificial Sequence
  source: /note="Description of Artificial Sequence: Synthetic peptide"
CATWDKPQIFYKKLF

SEQ ID NO: 331 - protein, 15 aa, Artificial Sequence
  source: /note="Description of Artificial Sequence: Synthetic peptide"
CATWEKPQIFYKKLF

SEQ ID NO: 332 - protein, 15 aa, Artificial Sequence
  source: /note="Description of Artificial Sequence: Synthetic peptide"
CATWNKPQIFYKKLF

SEQ ID NO: 333 - protein, 15 aa, Artificial Sequence
  source: /note="Description of Artificial Sequence: Synthetic peptide"
CATWQKPQIFYKKLF

SEQ ID NO: 334 - protein, 15 aa, Artificial Sequence
  source: /note="Description of Artificial Sequence: Synthetic peptide"
CATWDRPELFYKKLF

SEQ ID NO: 335 - protein, 15 aa, Artificial Sequence
  source: /note="Description of Artificial Sequence: Synthetic peptide"
CATWERPELFYKKLF

SEQ ID NO: 336 - protein, 15 aa, Artificial Sequence
  source: /note="Description of Artificial Sequence: Synthetic peptide"
CATWNRPELFYKKLF

SEQ ID NO: 337 - protein, 15 aa, Artificial Sequence
  source: /note="Description of Artificial Sequence: Synthetic peptide"
CATWQRPELFYKKLF

SEQ ID NO: 338 - protein, 15 aa, Artificial Sequence
  source: /note="Description of Artificial Sequence: Synthetic peptide"
CATWDKPELFYKKLF

SEQ ID NO: 339 - protein, 15 aa, Artificial Sequence
  source: /note="Description of Artificial Sequence: Synthetic peptide"
CATWEKPELFYKKLF

SEQ ID NO: 340 - protein, 15 aa, Artificial Sequence
  source: /note="Description of Artificial Sequence: Synthetic peptide"
CATWNKPELFYKKLF

SEQ ID NO: 341 - protein, 15 aa, Artificial Sequence
  source: /note="Description of Artificial Sequence: Synthetic peptide"
CATWQKPELFYKKLF

SEQ ID NO: 342 - protein, 15 aa, Artificial Sequence
  source: /note="Description of Artificial Sequence: Synthetic peptide"
CATWDRPDLFYKKLF

SEQ ID NO: 343 - protein, 15 aa, Artificial Sequence
  source: /note="Description of Artificial Sequence: Synthetic peptide"
CATWERPDLFYKKLF

SEQ ID NO: 344 - protein, 15 aa, Artificial Sequence
  source: /note="Description of Artificial Sequence: Synthetic peptide"
CATWNRPDLFYKKLF

SEQ ID NO: 345 - protein, 15 aa, Artificial Sequence
  source: /note="Description of Artificial Sequence: Synthetic peptide"
CATWQRPDLFYKKLF

SEQ ID NO: 346 - protein, 15 aa, Artificial Sequence
  source: /note="Description of Artificial Sequence: Synthetic peptide"
CATWDKPDLFYKKLF

SEQ ID NO: 347 - protein, 15 aa, Artificial Sequence
  source: /note="Description of Artificial Sequence: Synthetic peptide"
CATWEKPDLFYKKLF

SEQ ID NO: 348 - protein, 15 aa, Artificial Sequence
  source: /note="Description of Artificial Sequence: Synthetic peptide"
CATWNKPDLFYKKLF

SEQ ID NO: 349 - protein, 15 aa, Artificial Sequence
  source: /note="Description of Artificial Sequence: Synthetic peptide"
CATWQKPDLFYKKLF

SEQ ID NO: 350 - protein, 15 aa, Artificial Sequence
  source: /note="Description of Artificial Sequence: Synthetic peptide"
CATWDRPNLFYKKLF

SEQ ID NO: 351 - protein, 15 aa, Artificial Sequence
  source: /note="Description of Artificial Sequence: Synthetic peptide"
CATWERPNLFYKKLF

SEQ ID NO: 352 - protein, 15 aa, Artificial Sequence
  source: /note="Description of Artificial Sequence: Synthetic peptide"
CATWNRPNLFYKKLF

SEQ ID NO: 353 - protein, 15 aa, Artificial Sequence
  source: /note="Description of Artificial Sequence: Synthetic peptide"
CATWQRPNLFYKKLF

SEQ ID NO: 354 - protein, 15 aa, Artificial Sequence
  source: /note="Description of Artificial Sequence: Synthetic peptide"
CATWDKPNLFYKKLF

SEQ ID NO: 355 - protein, 15 aa, Artificial Sequence
  source: /note="Description of Artificial Sequence: Synthetic peptide"
CATWEKPNLFYKKLF

SEQ ID NO: 356 - protein, 15 aa, Artificial Sequence
  source: /note="Description of Artificial Sequence: Synthetic peptide"
CATWNKPNLFYKKLF

SEQ ID NO: 357 - protein, 15 aa, Artificial Sequence
  source: /note="Description of Artificial Sequence: Synthetic peptide"
CATWQKPNLFYKKLF

SEQ ID NO: 358 - protein, 15 aa, Artificial Sequence
  source: /note="Description of Artificial Sequence: Synthetic peptide"
CATWDRPQLFYKKLF

SEQ ID NO: 359 - protein, 15 aa, Artificial Sequence
  source: /note="Description of Artificial Sequence: Synthetic peptide"
CATWERPQLFYKKLF

SEQ ID NO: 360 - protein, 15 aa, Artificial Sequence
  source: /note="Description of Artificial Sequence: Synthetic peptide"
CATWNRPQLFYKKLF

SEQ ID NO: 361 - protein, 15 aa, Artificial Sequence
  source: /note="Description of Artificial Sequence: Synthetic peptide"
CATWQRPQLFYKKLF

SEQ ID NO: 362 - protein, 15 aa, Artificial Sequence
  source: /note="Description of Artificial Sequence: Synthetic peptide"
CATWDKPQLFYKKLF

SEQ ID NO: 363 - protein, 15 aa, Artificial Sequence
  source: /note="Description of Artificial Sequence: Synthetic peptide"
CATWEKPQLFYKKLF

SEQ ID NO: 364 - protein, 15 aa, Artificial Sequence
  source: /note="Description of Artificial Sequence: Synthetic peptide"
CATWNKPQLFYKKLF

SEQ ID NO: 365 - protein, 15 aa, Artificial Sequence
  source: /note="Description of Artificial Sequence: Synthetic peptide"
CATWQKPQLFYKKLF

SEQ ID NO: 366 - protein, 15 aa, Artificial Sequence
  source: /note="Description of Artificial Sequence: Synthetic peptide"
CATWERPEVFYKKLF

SEQ ID NO: 367 - protein, 15 aa, Artificial Sequence
  source: /note="Description of Artificial Sequence: Synthetic peptide"
CATWNRPEVFYKKLF

SEQ ID NO: 368 - protein, 15 aa, Artificial Sequence
  source: /note="Description of Artificial Sequence: Synthetic peptide"
CATWQRPEVFYKKLF

SEQ ID NO: 369 - protein, 15 aa, Artificial Sequence
  source: /note="Description of Artificial Sequence: Synthetic peptide"
CATWDKPEVFYKKLF

SEQ ID NO: 370 - protein, 15 aa, Artificial Sequence
  source: /note="Description of Artificial Sequence: Synthetic peptide"
CATWEKPEVFYKKLF

SEQ ID NO: 371 - protein, 15 aa, Artificial Sequence
  source: /note="Description of Artificial Sequence: Synthetic peptide"
CATWNKPEVFYKKLF

SEQ ID NO: 372 - protein, 15 aa, Artificial Sequence
  source: /note="Description of Artificial Sequence: Synthetic peptide"
CATWQKPEVFYKKLF

SEQ ID NO: 373 - protein, 15 aa, Artificial Sequence
  source: /note="Description of Artificial Sequence: Synthetic peptide"
CATWDRPDVFYKKLF

SEQ ID NO: 374 - protein, 15 aa, Artificial Sequence
  source: /note="Description of Artificial Sequence: Synthetic peptide"
CATWERPDVFYKKLF

SEQ ID NO: 375 - protein, 15 aa, Artificial Sequence
  source: /note="Description of Artificial Sequence: Synthetic peptide"
CATWNRPDVFYKKLF

SEQ ID NO: 376 - protein, 15 aa, Artificial Sequence
  source: /note="Description of Artificial Sequence: Synthetic peptide"
CATWQRPDVFYKKLF

SEQ ID NO: 377 - protein, 15 aa, Artificial Sequence
  source: /note="Description of Artificial Sequence: Synthetic peptide"
CATWDKPDVFYKKLF

SEQ ID NO: 378 - protein, 15 aa, Artificial Sequence
  source: /note="Description of Artificial Sequence: Synthetic peptide"
CATWEKPDVFYKKLF

SEQ ID NO: 379 - protein, 15 aa, Artificial Sequence
  source: /note="Description of Artificial Sequence: Synthetic peptide"
CATWNKPDVFYKKLF

SEQ ID NO: 380 - protein, 15 aa, Artificial Sequence
  source: /note="Description of Artificial Sequence: Synthetic peptide"
CATWQKPDVFYKKLF

SEQ ID NO: 381 - protein, 15 aa, Artificial Sequence
  source: /note="Description of Artificial Sequence: Synthetic peptide"
CATWDRPNVFYKKLF

SEQ ID NO: 382 - protein, 15 aa, Artificial Sequence
  source: /note="Description of Artificial Sequence: Synthetic peptide"
CATWERPNVFYKKLF

SEQ ID NO: 383 - protein, 15 aa, Artificial Sequence
  source: /note="Description of Artificial Sequence: Synthetic peptide"
CATWNRPNVFYKKLF

SEQ ID NO: 384 - protein, 15 aa, Artificial Sequence
  source: /note="Description of Artificial Sequence: Synthetic peptide"
CATWQRPNVFYKKLF

SEQ ID NO: 385 - protein, 15 aa, Artificial Sequence
  source: /note="Description of Artificial Sequence: Synthetic peptide"
CATWDKPNVFYKKLF

SEQ ID NO: 386 - protein, 15 aa, Artificial Sequence
  source: /note="Description of Artificial Sequence: Synthetic peptide"
CATWEKPNVFYKKLF

SEQ ID NO: 387 - protein, 15 aa, Artificial Sequence
  source: /note="Description of Artificial Sequence: Synthetic peptide"
CATWNKPNVFYKKLF

SEQ ID NO: 388 - protein, 15 aa, Artificial Sequence
  source: /note="Description of Artificial Sequence: Synthetic peptide"
CATWQKPNVFYKKLF

SEQ ID NO: 389 - protein, 15 aa, Artificial Sequence
  source: /note="Description of Artificial Sequence: Synthetic peptide"
CATWDRPQVFYKKLF

SEQ ID NO: 390 - protein, 15 aa, Artificial Sequence
  source: /note="Description of Artificial Sequence: Synthetic peptide"
CATWERPQVFYKKLF

SEQ ID NO: 391 - protein, 15 aa, Artificial Sequence
  source: /note="Description of Artificial Sequence: Synthetic peptide"
CATWNRPQVFYKKLF

SEQ ID NO: 392 - protein, 15 aa, Artificial Sequence
  source: /note="Description of Artificial Sequence: Synthetic peptide"
CATWQRPQVFYKKLF

SEQ ID NO: 393 - protein, 15 aa, Artificial Sequence
  source: /note="Description of Artificial Sequence: Synthetic peptide"
CATWDKPQVFYKKLF

SEQ ID NO: 394 - protein, 15 aa, Artificial Sequence
  source: /note="Description of Artificial Sequence: Synthetic peptide"
CATWEKPQVFYKKLF

SEQ ID NO: 395 - protein, 15 aa, Artificial Sequence
  source: /note="Description of Artificial Sequence: Synthetic peptide"
CATWNKPQVFYKKLF

SEQ ID NO: 396 - protein, 15 aa, Artificial Sequence
  source: /note="Description of Artificial Sequence: Synthetic peptide"
CATWQKPQVFYKKLF

SEQ ID NO: 397 - protein, 15 aa, Artificial Sequence
  source: /note="Description of Artificial Sequence: Synthetic peptide"
CATWERPEVYYKKLF

SEQ ID NO: 398 - protein, 15 aa, Artificial Sequence
  source: /note="Description of Artificial Sequence: Synthetic peptide"
CATWNRPEVYYKKLF

SEQ ID NO: 399 - protein, 15 aa, Artificial Sequence
  source: /note="Description of Artificial Sequence: Synthetic peptide"
CATWQRPEVYYKKLF

SEQ ID NO: 400 - protein, 15 aa, Artificial Sequence
  source: /note="Description of Artificial Sequence: Synthetic peptide"
CATWDKPEVYYKKLF

SEQ ID NO: 401 - protein, 15 aa, Artificial Sequence
  source: /note="Description of Artificial Sequence: Synthetic peptide"
CATWEKPEVYYKKLF

SEQ ID NO: 402 - protein, 15 aa, Artificial Sequence
  source: /note="Description of Artificial Sequence: Synthetic peptide"
CATWNKPEVYYKKLF

SEQ ID NO: 403 - protein, 15 aa, Artificial Sequence
  source: /note="Description of Artificial Sequence: Synthetic peptide"
CATWQKPEVYYKKLF

SEQ ID NO: 404 - protein, 15 aa, Artificial Sequence
  source: /note="Description of Artificial Sequence: Synthetic peptide"
CATWDRPDVYYKKLF

SEQ ID NO: 405 - protein, 15 aa, Artificial Sequence
  source: /note="Description of Artificial Sequence: Synthetic peptide"
CATWERPDVYYKKLF

SEQ ID NO: 406 - protein, 15 aa, Artificial Sequence
  source: /note="Description of Artificial Sequence: Synthetic peptide"
CATWNRPDVYYKKLF

SEQ ID NO: 407 - protein, 15 aa, Artificial Sequence
  source: /note="Description of Artificial Sequence: Synthetic peptide"
CATWQRPDVYYKKLF

SEQ ID NO: 408 - protein, 15 aa, Artificial Sequence
  source: /note="Description of Artificial Sequence: Synthetic peptide"
CATWDKPDVYYKKLF

SEQ ID NO: 409 - protein, 15 aa, Artificial Sequence
  source: /note="Description of Artificial Sequence: Synthetic peptide"
CATWEKPDVYYKKLF

SEQ ID NO: 410 - protein, 15 aa, Artificial Sequence
  source: /note="Description of Artificial Sequence: Synthetic peptide"
CATWNKPDVYYKKLF

SEQ ID NO: 411 - protein, 15 aa, Artificial Sequence
  source: /note="Description of Artificial Sequence: Synthetic peptide"
CATWQKPDVYYKKLF

SEQ ID NO: 412 - protein, 15 aa, Artificial Sequence
  source: /note="Description of Artificial Sequence: Synthetic peptide"
CATWDRPNVYYKKLF

SEQ ID NO: 413 - protein, 15 aa, Artificial Sequence
  source: /note="Description of Artificial Sequence: Synthetic peptide"
CATWERPNVYYKKLF

SEQ ID NO: 414 - protein, 15 aa, Artificial Sequence
  source: /note="Description of Artificial Sequence: Synthetic peptide"
CATWNRPNVYYKKLF

SEQ ID NO: 415 - protein, 15 aa, Artificial Sequence
  source: /note="Description of Artificial Sequence: Synthetic peptide"
CATWQRPNVYYKKLF

SEQ ID NO: 416 - protein, 15 aa, Artificial Sequence
  source: /note="Description of Artificial Sequence: Synthetic peptide"
CATWDKPNVYYKKLF

SEQ ID NO: 417 - protein, 15 aa, Artificial Sequence
  source: /note="Description of Artificial Sequence: Synthetic peptide"
CATWEKPNVYYKKLF

SEQ ID NO: 418 - protein, 15 aa, Artificial Sequence
  source: /note="Description of Artificial Sequence: Synthetic peptide"
CATWNKPNVYYKKLF

SEQ ID NO: 419 - protein, 15 aa, Artificial Sequence
  source: /note="Description of Artificial Sequence: Synthetic peptide"
CATWQKPNVYYKKLF

SEQ ID NO: 420 - protein, 15 aa, Artificial Sequence
  source: /note="Description of Artificial Sequence: Synthetic peptide"
CATWDRPQVYYKKLF

SEQ ID NO: 421 - protein, 15 aa, Artificial Sequence
  source: /note="Description of Artificial Sequence: Synthetic peptide"
CATWERPQVYYKKLF

SEQ ID NO: 422 - protein, 15 aa, Artificial Sequence
  source: /note="Description of Artificial Sequence: Synthetic peptide"
CATWNRPQVYYKKLF

SEQ ID NO: 423 - protein, 15 aa, Artificial Sequence
  source: /note="Description of Artificial Sequence: Synthetic peptide"
CATWQRPQVYYKKLF

SEQ ID NO: 424 - protein, 15 aa, Artificial Sequence
  source: /note="Description of Artificial Sequence: Synthetic peptide"
CATWDKPQVYYKKLF

SEQ ID NO: 425 - protein, 15 aa, Artificial Sequence
  source: /note="Description of Artificial Sequence: Synthetic peptide"
CATWEKPQVYYKKLF

SEQ ID NO: 426 - protein, 15 aa, Artificial Sequence
  source: /note="Description of Artificial Sequence: Synthetic peptide"
CATWNKPQVYYKKLF

SEQ ID NO: 427 - protein, 15 aa, Artificial Sequence
  source: /note="Description of Artificial Sequence: Synthetic peptide"
CATWQKPQVYYKKLF

SEQ ID NO: 428 - protein, 13 aa, Artificial Sequence
  source: /note="Description of Artificial Sequence: Synthetic peptide"
ATWDRPEIYYKKL

SEQ ID NO: 429 - DNA, 20 bp, Artificial Sequence
  source: /note="Description of Artificial Sequence: Synthetic primer"
gatcaagtgtggcccagaag

SEQ ID NO: 430 - DNA, 20 bp, Artificial Sequence
  source: /note="Description of Artificial Sequence: Synthetic primer"
ctgccagtcagaaatcttcc

SEQ ID NO: 431 - DNA, 18 bp, Artificial Sequence
  source: /note="Description of Artificial Sequence: Synthetic primer"
ttcaccagacaagcgaca

SEQ ID NO: 432 - DNA, 18 bp, Artificial Sequence
  source: /note="Description of Artificial Sequence: Synthetic primer"
ggggaaacatctgcatca

SEQ ID NO: 433 - protein, 9 aa, Artificial Sequence
  source: /note="Description of Artificial Sequence: Synthetic peptide"
SLLMWITQV

SEQ ID NO: 434 - protein, 9 aa, Artificial Sequence
  source: /note="Description of Artificial Sequence: Synthetic peptide"
QYDPVAALF

SEQ ID NO: 435 - protein, 9 aa, Homo sapiens
RMFPNAPYL

SEQ ID NO: 436 - DNA, 20 bp, Artificial Sequence
  source: /note="Description of Artificial Sequence: Synthetic oligonucleotide"
gagtagcgcgagcacagcta

SEQ ID NO: 437 - DNA, 20 bp, Artificial Sequence
  source: /note="Description of Artificial Sequence: Synthetic oligonucleotide"
ggagcgcaccatcttcttca

SEQ ID NO: 438 - protein, 10 aa, Artificial Sequence
  source: /note="Description of Artificial Sequence: Synthetic peptide"
RYPLTFGWCF

SEQ ID NO: 439 - protein, 350 aa, Homo sapiens
MAVMAPRTLVLLLSGALALTQTWAGSHSMRYFFTSVSRPGRGEPRFIAVGYVDDTQFVRFDSDAASQRMEPRAPWIEQEGPEYWDGETRKVKAHSQTHRVDLGTLRGYYNQSEAGSHTVQRMYGCDVGSDWRFLRGYHQYAYDGKDYIALKEDLRSWTAADMAAQTTKHKWEAAHVAEQLRAYLEGTCVEWLRRYLENGKETLQRTDAPKTHMTHHAVSDHEATLRCWALSFYPAEITLTWQRDGEDQTQDTELVETRPAGDGTFQKWAAVVVPSGQEQRYTCHVQHEGLPKPLTLRWEPSSQPTIPIVGIIAGLVLFGAVITGAVVAAVMWRRKSSDRKGGSYSQAASS

SEQ ID NO: 440 - protein, 350 aa, Homo sapiens
MAVMAPRTLVLLLSGALALTQTWAGSHSMRYFSTSVSRPGRGEPRFIAVGYVDDTQFVRFDSDAASQRMEPRAPWIEQEGPEYWDEETGKVKAHSQTDRENLRIALRYYNQSEAGSHTLQMMFGCDVGSDGRFLRGYHQYAYDGKDYIALKEDLRSWTAADMAAQITKRKWEAAHVAEQQRAYLEGTCVDGLRRYLENGKETLQRTDPPKTHMTHHPISDHEATLRCWALGFYPAEITLTWQRDGEDQTQDTELVETRPAGDGTFQKWAAVVVPSGEEQRYTCHVQHEGLPKPLTLRWEPSSQPTVPIVGIIAGLVLLGAVITGAVVAAVMWRRNSSDRKGGSYSQAASS

SEQ ID NO: 441 - protein, 30 aa, Homo sapiens
HVAEQQRAYLEGTCVDGLRRYLENGKETLQ

SEQ ID NO: 442 - protein, 30 aa, Homo sapiens
HVAEQLRAYLEGTCVEWLRRYLENGKETLQ

SEQ ID NO: 443 - protein, 30 aa, Homo sapiens
HVAEQQRAYLEGTCVEWLRRYLENGKETLQ

SEQ ID NO: 444 - protein, 30 aa, Homo sapiens
HEAEQWRAYLEGRCVEWLRRYLENGKETLQ